European Patent Application EP 4 495 257 A1, published January 22, 2025. Title: 단일 염기 다형성 분석을 위한 미세입자 프로브. Applicant: 주식회사 이지다디아텍. Application KR. The sequence listing filed with the application follows.

SEQUENCE LISTING (6 sequences)

SEQ ID NO: 1 - DNA, 25 bp, synthetic construct
  source 1..25: mol_type = other DNA
aagagaaagacctccctttgggcaa

SEQ ID NO: 2 - DNA, 25 bp, synthetic construct
  source 1..25: mol_type = other DNA
cacccctgatggtgctatcgacaag

SEQ ID NO: 3 - RNA, 40 nt, synthetic construct
  source 1..40: mol_type = other RNA
taatttctactaagtgtagatcattgtctcaccgatacac

SEQ ID NO: 4 - RNA, 40 nt, synthetic construct
  source 1..40: mol_type = other RNA
taatttctactaagtgtagatcactgtctcaccgatacac

SEQ ID NO: 5 - skipped

SEQ ID NO: 6 - DNA, 10 bp, synthetic construct
  source 1..10: mol_type = other DNA
ttattatttt